European Patent Specification EP 3 740 755 B9, published October 4, 2023. Title: Use of the TAS1R3 protein as a marker for therapeutic, diagnostic, and/or prognostic purposes for tumors that express said protein. Applicant: FUNDACIÓN PARA A INVESTIGACIÓN, DESENVOLVEMENTO E INNOVACIÓN RAMÓN DOMÍNGUEZ SERVIZO GALEGO DE SAÚDE. Application EP18382013.3. The sequence listing filed with the application follows.

SEQUENCE LISTING (3 sequences)

SEQ ID NO: 1 - protein, 16 aa, Artificial Sequence
  MOD_RES 1: acetyllysine ACETYLATION
  synthetic peptide
  MOD_RES 16: cysteinamide
LSQQLRMKGDYVLGGC

SEQ ID NO: 2 - protein, 19 aa, Artificial Sequence
  MOD_RES 1: acetylglutamic acid ACETYLATION
  synthetic peptide
  MOD_RES 19: cysteinamide AMIDATION
ERLKIRWHTSDNQKPVSRC

SEQ ID NO: 3 - protein, 7 aa, Artificial Sequence
  BRA
CFYDEKR